European Patent Application EP 4 692 372 A1, published February 11, 2026. Title: UNIVERSAL LANDING PLATFORM. Applicant: UNIVERCELLS FRANCE SAS. Application EP. The sequence listing filed with the application follows.

SEQUENCE LISTING (57 sequences)

SEQ ID NO: 1 - DNA, 26 bp, synthetic construct
  source 1..26: mol_type = other DNA
gvdnhnsrknhbcdmctbmrbysgrc

SEQ ID NO: 2 - DNA, 26 bp, synthetic construct
  source 1..26: mol_type = other DNA
gvdnhnsrknhbckmctbmastcggc

SEQ ID NO: 3 - DNA, 26 bp, synthetic construct
  source 1..26: mol_type = other DNA
garrmssakwyscrccnnngtyggan

SEQ ID NO: 4 - DNA, 26 bp, synthetic construct
  source 1..26: mol_type = other DNA
gagacccagttccgcctgcactcggc

SEQ ID NO: 5 - DNA, 26 bp, synthetic construct
  source 1..26: mol_type = other DNA
gagacccagttccgcctcaagnnnnn

SEQ ID NO: 6 - DNA, 26 bp, synthetic construct
  source 1..26: mol_type = other DNA
gagacccagtnccacnnnngttggan

SEQ ID NO: 7 - DNA, 26 bp, synthetic construct
  source 1..26: mol_type = other DNA
ncactgcnnntccgcctgcactcggc

SEQ ID NO: 8 - DNA, 26 bp, synthetic construct
  source 1..26: mol_type = other DNA
ncactgcnncatcgcctgcactcggc

SEQ ID NO: 9 - DNA, 26 bp, synthetic construct
  source 1..26: mol_type = other DNA
gaagagnnnctcctcctgcactcggc

SEQ ID NO: 10 - DNA, 26 bp, synthetic construct
  source 1..26: mol_type = other DNA
gagacccagtngntacttcagtnnnn

SEQ ID NO: 11 - DNA, 26 bp, synthetic construct
  source 1..26: mol_type = other DNA
gagacccagtngcannnnngtcggan

SEQ ID NO: 12 - DNA, 26 bp, synthetic construct
  source 1..26: mol_type = other DNA
gagaccnnnntccgcctgcactcggc

SEQ ID NO: 13 - DNA, 26 bp, synthetic construct
  source 1..26: mol_type = other DNA
gagacccagttccgcctgcacnnnnn

SEQ ID NO: 14 - DNA, 26 bp, synthetic construct
  source 1..26: mol_type = other DNA
ncactgcnnctcctcctgcactcggc

SEQ ID NO: 15 - DNA, 26 bp, synthetic construct
  source 1..26: mol_type = other DNA
gcattcnnnctcctcctgcactcggc

SEQ ID NO: 16 - DNA, 26 bp, synthetic construct
  source 1..26: mol_type = other DNA
gaagagcnnntccgcctgcactcggc

SEQ ID NO: 17 - DNA, 26 bp, synthetic construct
  source 1..26: mol_type = other DNA
gaagaggatacgntacttcagtnnnn

SEQ ID NO: 18 - DNA, 26 bp, synthetic construct
  source 1..26: mol_type = other DNA
gaagagcnnctcctcctgcactcggc

SEQ ID NO: 19 - DNA, 26 bp, synthetic construct
  source 1..26: mol_type = other DNA
gagacggatacgntactccagtnnnn

SEQ ID NO: 20 - DNA, 26 bp, synthetic construct
  source 1..26: mol_type = other DNA
nnnncccagttccgcctgcactcggc

SEQ ID NO: 21 - DNA, 26 bp, synthetic construct
  source 1..26: mol_type = other DNA
gagacccagtngntactccagtnnnn

SEQ ID NO: 22 - DNA, 26 bp, synthetic construct
  source 1..26: mol_type = other DNA
gaagaggatacgntactcaagtnnnn

SEQ ID NO: 23 - DNA, 26 bp, synthetic construct
  source 1..26: mol_type = other DNA
gagacggatacnnnnctgcactcggc

SEQ ID NO: 24 - DNA, 26 bp, synthetic construct
  source 1..26: mol_type = other DNA
ncattgcnnctcctcctgcactcggc

SEQ ID NO: 25 - DNA, 26 bp, synthetic construct
  source 1..26: mol_type = other DNA
gcattcnnncatcgcctgcactcggc

SEQ ID NO: 26 - DNA, 26 bp, synthetic construct
  source 1..26: mol_type = other DNA
ngtcttcnnctcctcctgcactcggc

SEQ ID NO: 27 - DNA, 26 bp, synthetic construct
  source 1..26: mol_type = other DNA
gaagagnnnntccgcctgcactcggc

SEQ ID NO: 28 - DNA, 26 bp, synthetic construct
  source 1..26: mol_type = other DNA
gagacgnnnntccgcctgcactcggc

SEQ ID NO: 29 - DNA, 26 bp, synthetic construct
  source 1..26: mol_type = other DNA
nnngcaggtgtccgcctgcactcggc

SEQ ID NO: 30 - DNA, 26 bp, synthetic construct
  source 1..26: mol_type = other DNA
gagaccnnnctcctcctgcactcggc

SEQ ID NO: 31 - DNA, 26 bp, synthetic construct
  source 1..26: mol_type = other DNA
gagacccagtnnnnnctgcactcggc

SEQ ID NO: 32 - DNA, 26 bp, synthetic construct
  source 1..26: mol_type = other DNA
gagacccagttccgccnnnnctcggc

SEQ ID NO: 33 - DNA, 26 bp, synthetic construct
  source 1..26: mol_type = other DNA
gcattcnnnntccgcctgcactcggc

SEQ ID NO: 34 - DNA, 26 bp, synthetic construct
  source 1..26: mol_type = other DNA
gagacgnnnctcctcctgcactcggc

SEQ ID NO: 35 - DNA, 26 bp, synthetic construct
  source 1..26: mol_type = other DNA
gaagagnnncatcgcctgcactcggc

SEQ ID NO: 36 - DNA, 26 bp, synthetic construct
  source 1..26: mol_type = other DNA
gagacgnnncatcgcctgcactcggc

SEQ ID NO: 37 - DNA, 26 bp, synthetic construct
  source 1..26: mol_type = other DNA
gagacggatacgntacttcagtnnnn

SEQ ID NO: 38 - DNA, 26 bp, synthetic construct
  source 1..26: mol_type = other DNA
ncattgcnnntccgcctgcactcggc

SEQ ID NO: 39 - DNA, 26 bp, synthetic construct
  source 1..26: mol_type = other DNA
nnngcaggtctcctcctgcactcggc

SEQ ID NO: 40 - DNA, 26 bp, synthetic construct
  source 1..26: mol_type = other DNA
gagacggatacccacnnnngttggan

SEQ ID NO: 41 - DNA, 26 bp, synthetic construct
  source 1..26: mol_type = other DNA
gagaccnnncatcgcctgcactcggc

SEQ ID NO: 42 - DNA, 26 bp, synthetic construct
  source 1..26: mol_type = other DNA
ngtcttcnncatcgcctgcactcggc

SEQ ID NO: 43 - DNA, 26 bp, synthetic construct
  source 1..26: mol_type = other DNA
gaagaggatacnnnnctgcactcggc

SEQ ID NO: 44 - DNA, 26 bp, synthetic construct
  source 1..26: mol_type = other DNA
gagacccagtngntactcaagtnnnn

SEQ ID NO: 45 - DNA, 26 bp, synthetic construct
  source 1..26: mol_type = other DNA
gaagaggatacgntactccagtnnnn

SEQ ID NO: 46 - DNA, 26 bp, synthetic construct
  source 1..26: mol_type = other DNA
gaagaggatacccacnnnngttggan

SEQ ID NO: 47 - DNA, 26 bp, synthetic construct
  source 1..26: mol_type = other DNA
ngtcttcnnntccgcctgcactcggc

SEQ ID NO: 48 - DNA, 26 bp, synthetic construct
  source 1..26: mol_type = other DNA
ncattgcnncatcgcctgcactcggc

SEQ ID NO: 49 - DNA, 26 bp, synthetic construct
  source 1..26: mol_type = other DNA
gagacccagttccgccnnngtnggan

SEQ ID NO: 50 - DNA, 26 bp, synthetic construct
  source 1..26: mol_type = other DNA
gagacccagttccgccttcagnnnnn

SEQ ID NO: 51 - DNA, 26 bp, synthetic construct
  source 1..26: mol_type = other DNA
nnngcaggtcatcgcctgcactcggc

SEQ ID NO: 52 - DNA, 26 bp, synthetic construct
  source 1..26: mol_type = other DNA
gaagaggatacgcannnnngtcggan

SEQ ID NO: 53 - DNA, 26 bp, synthetic construct
  source 1..26: mol_type = other DNA
gaagagcnncatcgcctgcactcggc

SEQ ID NO: 54 - DNA, 26 bp, synthetic construct
  source 1..26: mol_type = other DNA
nnngcaggtntccgcctgcactcggc

SEQ ID NO: 55 - DNA, 26 bp, synthetic construct
  source 1..26: mol_type = other DNA
gagacggatacgcannnnngtcggan

SEQ ID NO: 56 - DNA, 26 bp, synthetic construct
  source 1..26: mol_type = other DNA
gagacggatacgntactcaagtnnnn

SEQ ID NO: 57 - DNA, 26 bp, synthetic construct
  source 1..26: mol_type = other DNA
gagacccagttccgcctccagnnnnn